European Patent Specification EP 3 572 511 B1, published July 12, 2023. Title: Complex containing Oligonucleotide having immunopotentiating activity and use thereof. Applicant: National Institutes of Biomedical Innovation, Health and Nutrition Daiichi Sankyo Company, Limited. Application EP 14846493.6. The sequence listing filed with the application follows.

SEQUENCE LISTING (15 sequences)

SEQ ID NO: 1 - DNA, 20 bp, Artificial Sequence
  Synthetic Oligonucleotide
atcgactctcgagcgttctc

SEQ ID NO: 2 - DNA, 60 bp, Artificial Sequence
  Synthetic Oligonucleotide
atcgactctcgagcgttctcaaaaaaaaaaaaaaaaaaaaaaaaaaaaaaaaaaaaaaaa

SEQ ID NO: 3 - DNA, 60 bp, Artificial Sequence
  Synthetic Oligonucleotide
aaaaaaaaaaaaaaaaaaaaaaaaaaaaaaaaaaaaaaaaatcgactctcgagcgttctc

SEQ ID NO: 4 - DNA, 20 bp, Artificial Sequence
  Synthetic Oligonucleotide
ggtgcatcgatgcagggggg

SEQ ID NO: 5 - DNA, 23 bp, Artificial Sequence
  Synthetic Oligonucleotide
tcgtcgacgatcggcgcgcgccg

SEQ ID NO: 6 - DNA, 23 bp, Artificial Sequence
  Synthetic Oligonucleotide
tcgtcgacgatcggcgcgcgccg

SEQ ID NO: 7 - DNA, 22 bp, Artificial Sequence
  Synthetic Oligonucleotide
tcgtcgttttcggcgcgcgccg

SEQ ID NO: 8 - DNA, 25 bp, Artificial Sequence
  Synthetic Oligonucleotide
tcgtcgtcgttcgaacgacgttgat

SEQ ID NO: 9 - DNA, 40 bp, Artificial Sequence
  Synthetic Oligonucleotide
atcgactctcgagcgttctcaaaaaaaaaaaaaaaaaaaa

SEQ ID NO: 10 - DNA, 45 bp, Artificial Sequence
  Synthetic Oligonucleotide
atcgactctcgagcgttctcaaaaaaaaaaaaaaaaaaaaaaaaa

SEQ ID NO: 11 - DNA, 50 bp, Artificial Sequence
  Synthetic Oligonucleotide
atcgactctcgagcgttctcaaaaaaaaaaaaaaaaaaaaaaaaaaaaaa

SEQ ID NO: 12 - DNA, 55 bp, Artificial Sequence
  Synthetic Oligonucleotide
atcgactctcgagcgttctcaaaaaaaaaaaaaaaaaaaaaaaaaaaaaaaaaaa

SEQ ID NO: 13 - protein, 8 aa, Unknown
  OVA257
SIINFEKL

SEQ ID NO: 14 - protein, 17 aa, Unknown
  OVA323
ISQAVHAAHAEINEAGR

SEQ ID NO: 15 - protein, 24 aa, Unknown
  NP260
ARSALILRGSVAHKSCLPACVYGP